European Patent Application EP 4 772 636 A1, published July 8, 2026. Title: T细胞激活后特异诱导基因表达的重组启动子系统. Applicant: 徐州医科大学. The sequence listing filed with the application follows.

SEQUENCE LISTING (31 sequences)

SEQ ID NO: 1 - DNA, 720 bp, synthetic construct
  source 1..720: mol_type = other DNA; note = 376.96 scFv
gacattgtgatgacccagtctcacaaattcatgtccacatcaattggagccagggtcagcatcacctgcaaggccagtcaggatgtgagaactgctgtagcctggtatcaacagaaaccaggccagtctcctaaactactaatttactcggcatcctaccggtacactggagtccctgatcgcttcactggcagtggatctgggacggatttcactttcaccatcagcagtgtgcaggctgaagacctggcagtttattactgtcagcaacattatggtactcctccgtggacgttcggtggaggcaccaagctggaaatcaaaggcggcggaggatctggcggaggcggaagtggcggagggggctctgaagtgcagctggtggagtctgggggaggcttagtgaagcctggagggtccctgaaactctcctgtgaagcctctagattcactttcagtagctatgccatgtcttgggttcgccagactccggagaagaggctggagtgggtcgcagccattagtggaggtggtaggtacacctactatccagacagtatgaagggtcgattcaccatctccagagacaatgccaagaatttcctgtacctgcaaatgagcagtctgaggtctgaggacacggccatgtattactgtgcaagacactatgatggttatcttgactactggggccaaggcaccactctcacagtctcctca

SEQ ID NO: 2 - protein, 240 aa, synthetic construct
  source 1..240: note = 376.96 scFv
DIVMTQSHKFMSTSIGARVSITCKASQDVRTAVAWYQQKPGQSPKLLIYSASYRYTGVPDRFTGSGSGTDFTFTISSVQAEDLAVYYCQQHYGTPPWTFGGGTKLEIKGGGGSGGGGSGGGGSEVQLVESGGGLVKPGGSLKLSCEASRFTFSSYAMSWVRQTPEKRLEWVAAISGGGRYTYYPDSMKGRFTISRDNAKNFLYLQMSSLRSEDTAMYYCARHYDGYLDYWGQGTTLTVSS

SEQ ID NO: 3 - DNA, 207 bp, Homo sapiens
  source 1..207: mol_type = genomic DNA
accacgacgccagcgccgcgaccaccaacaccggcgcccaccatcgcgtcgcagcccctgtccctgcgcccagaggcgtgccggccagcggcggggggcgcagtgcacacgagggggctggacttcgcctgtgatatctacatctgggcgcccttggccgggacttgtggggtccttctcctgtcactggttatcaccctttactgc

SEQ ID NO: 4 - protein, 69 aa, Homo sapiens
TTTPAPRPPTPAPTIASQPLSLRPEACRPAAGGAVHTRGLDFACDIYIWAPLAGTCGVLLLSLVITLYC

SEQ ID NO: 5 - DNA, 123 bp, Homo sapiens
  source 1..123: mol_type = genomic DNA
aggagtaagaggagcaggctcctgcacagtgactacatgaacatgactccccgccgccccgggcccacccgcaagcattaccagccctatgccccaccacgcgacttcgcagcctatcgctcc

SEQ ID NO: 6 - protein, 41 aa, Homo sapiens
RSKRSRLLHSDYMNMTPRRPGPTRKHYQPYAPPRDFAAYRS

SEQ ID NO: 7 - DNA, 336 bp, Homo sapiens
  source 1..336: mol_type = genomic DNA
agagtgaagttcagcaggagcgcagacgcccccgcgtaccagcagggccagaaccagctctataacgagctcaatctaggacgaagagaggagtacgatgttttggacaagagacgtggccgggaccctgagatggggggaaagccgagaaggaagaaccctcaggaaggcctgtacaatgaactgcagaaagataagatggcggaggcctacagtgagattgggatgaaaggcgagcgccggaggggcaaggggcacgatggcctttaccagggtctcagtacagccaccaaggacacctacgacgcccttcacatgcaggccctgccccctcgc

SEQ ID NO: 8 - protein, 112 aa, Homo sapiens
RVKFSRSADAPAYQQGQNQLYNELNLGRREEYDVLDKRRGRDPEMGGKPRRKNPQEGLYNELQKDKMAEAYSEIGMKGERRRGKGHDGLYQGLSTATKDTYDALHMQALPPR

SEQ ID NO: 9 - DNA, 510 bp, Mus musculus
  source 1..510: mol_type = genomic DNA
atgtacagcatgcagctcgcatcctgtgtcacattgacacttgtgctccttgtcaacagcgcacccacttcaagctccacttcaagctctacagcggaagcacagcagcagcagcagcagcagcagcagcagcagcagcacctggagcagctgttgatggacctacaggagctcctgagcaggatggagaattacaggaacctgaaactccccaggatgctcaccttcaaattttacttgcccaagcaggccacagaattgaaagatcttcagtgcctagaagatgaacttggacctctgcggcatgttctggatttgactcaaagcaaaagctttcaattggaagatgctgagaatttcatcagcaatatcagagtaactgttgtaaaactaaagggctctgacaacacatttgagtgccaattcgatgatgagtcagcaactgtggtggactttctgaggagatggatagccttctgtcaaagcatcatctcaacaagccctcaataa

SEQ ID NO: 10 - protein, 169 aa, Mus musculus
MYSMQLASCVTLTLVLLVNSAPTSSSTSSSTAEAQQQQQQQQQQQQHLEQLLMDLQELLSRMENYRNLKLPRMLTFKFYLPKQATELKDLQCLEDELGPLRHVLDLTQSKSFQLEDAENFISNIRVTVVKLKGSDNTFECQFDDESATVVDFLRRWIAFCQSIISTSPQ

SEQ ID NO: 11 - DNA, 372 bp, synthetic construct
  source 1..372: mol_type = other DNA; note = pGM-CSF Fragment
taagtgtctcccacgccccaccccagccattccaggccaggaagtccaaactgtgcccctcagagggagggggcagcctcaggcccattcagactgcccagggagggctggagagccctcaggaaggcgggtgggtgggctgtcggttcttggaaaggttcattaatgaaaacccccaagcctgaccacctagggaaaaggctcaccgttcccatgtgtggctgataagggccaggagattccacagttcaggtagttcccccgcctccctggcattttgtggtcaccattaatcatttcctctgtgtatttaagagctcttttgccagtgagcccagtacacagagagaaaggctaaagttctctggagga

SEQ ID NO: 12 - DNA, 336 bp, synthetic construct
  source 1..336: mol_type = other DNA; note = pGM-CSF Fragment
taagtgtctcccacgccccaccccagccattccaggccaggaagtccaaactgtgcccctcagagggagggggcagcctcaggcccattcagactgcccagggagggctggagagccctcaggaaggcgggtgggtgggctgtcggttcttggaaaggttcattaatgaaaacccccaagcctgaccacctagggaaaaggctcaccgttcccatgtgtggctgataagggccaggagattccacagttcaggtagttcccccgcctccctggcattttgtggtcaccattaatcatttcctctgtgtatttaagagctcttttgccagtgagccc

SEQ ID NO: 13 - DNA, 302 bp, synthetic construct
  source 1..302: mol_type = other DNA; note = pGM-CSF Fragment
taagtgtctcccacgccccaccccagccattccaggccaggaagtccaaactgtgcccctcagagggagggggcagcctcaggcccattcagactgcccagggagggctggagagccctcaggaaggcgggtgggtgggctgtcggttcttggaaaggttcattaatgaaaacccccaagcctgaccacctagggaaaaggctcaccgttcccatgtgtggctgataagggccaggagattccacagttcaggtagttcccccgcctccctggcattttgtggtcaccattaatcatttcct

SEQ ID NO: 14 - DNA, 253 bp, synthetic construct
  source 1..253: mol_type = other DNA; note = pGM-CSF Fragment
caggaaggcgggtgggtgggctgtcggttcttggaaaggttcattaatgaaaacccccaagcctgaccacctagggaaaaggctcaccgttcccatgtgtggctgataagggccaggagattccacagttcaggtagttcccccgcctccctggcattttgtggtcaccattaatcatttcctctgtgtatttaagagctcttttgccagtgagcccagtacacagagagaaaggctaaagttctctggagga

SEQ ID NO: 15 - DNA, 217 bp, synthetic construct
  source 1..217: mol_type = other DNA; note = pGM-CSF Fragment
caggaaggcgggtgggtgggctgtcggttcttggaaaggttcattaatgaaaacccccaagcctgaccacctagggaaaaggctcaccgttcccatgtgtggctgataagggccaggagattccacagttcaggtagttcccccgcctccctggcattttgtggtcaccattaatcatttcctctgtgtatttaagagctcttttgccagtgagccc

SEQ ID NO: 16 - DNA, 183 bp, synthetic construct
  source 1..183: mol_type = other DNA; note = pGM-CSF Fragment
caggaaggcgggtgggtgggctgtcggttcttggaaaggttcattaatgaaaacccccaagcctgaccacctagggaaaaggctcaccgttcccatgtgtggctgataagggccaggagattccacagttcaggtagttcccccgcctccctggcattttgtggtcaccattaatcatttcct

SEQ ID NO: 17 - DNA, 662 bp, synthetic construct
  source 1..662: mol_type = other DNA; note = pGM-CSF Fragment
gcttgctgagagtggctgcagtctcgctgctggatgtgcacatggtggtcattccctctgctcacaggggcaggggtccccccttactggactgaggttgccccctgctccaggtcctgggtgggagcccatgtgaactgtcagtggggcaggtctgtgagagctcccctcacactcaagtctctcacagtggccagagaagaggaaggctggagtcagaatgaggcaccagggcgggcatagcctgcccaaaggcccctgggattacaggcaggatggggagccctatctaagtgtctcccacgccccaccccagccattccaggccaggaagtccaaactgtgcccctcagagggagggggcagcctcaggcccattcagactgcccagggagggctggagagccctcaggaaggcgggtgggtgggctgtcggttcttggaaaggttcattaatgaaaacccccaagcctgaccacctagggaaaaggctcaccgttcccatgtgtggctgataagggccaggagattccacagttcaggtagttcccccgcctccctggcattttgtggtcaccattaatcatttcctctgtgtatttaagagctcttttgccagtgagcccagtacacagagagaaaggctaaagttctctggagga

SEQ ID NO: 18 - DNA, 373 bp, synthetic construct
  source 1..373: mol_type = other DNA; note = pIL2 Fragment
ttttctgagttacttttgtatccccacccccttaaagaaaggaggaaaaactgtttcatacagaaggcgttaattgcatgaattagagctatcacctaagtgtgggctaatgtaacaaagagggatttcacctacatccattcagtcagtctttgggggtttaaagaaattccaaagagtcatcagaagaggaaaaatgaaggtaatgttttttcagacaggtaaagtctttgaaaatatgtgtaatatgtaaaacattttgacacccccataatatttttccagaattaacagtataaattgcatctcttgttcaagagttccctatcactctctttaatcactactcacagtaacctcaactcctgccaca

SEQ ID NO: 19 - DNA, 602 bp, synthetic construct
  source 1..602: mol_type = other DNA; note = pIFN Fragment
tagagcaatttgaaacttgtggtagatattttactaaccaactctgatgaaggacttcctcaccaaattgttcttttaaccgcattctttccttgctttctggtcatttgcaagaaaaattttaaaaggctgcccctttgtaaaggtttgagaggccctagaatttcgtttttcacttgttcccaaccacaagcaaatgatcaatgtgctttgtgaatgaagagtcaacattttaccagggcgaagtggggaggtacaaaaaaatttccagtccttgaatggtgtgaagtaaaagtgccttcaaagaatcccaccagaatggcacaggtgggcataatgggtctgtctcatcgtcaaaggacccaaggagtctaaaggaaactctaactacaacacccaaatgccacaaaaccttagttattaatacaaactatcatccctgcctatctgtcaccatctcatcttaaaaaacttgtgaaaatacgtaatcctcaggagacttcaattaggtataaataccagcagccagaggaggtgcagcacattgttctgatcatctgaagatcagctattagaagagaaagatcagttaagtcctttgg

SEQ ID NO: 20 - DNA, 172 bp, synthetic construct
  source 1..172: mol_type = other DNA; note = pIFN Fragment
ctatcatccctgcctatctgtcaccatctcatcttaaaaaacttgtgaaaatacgtaatcctcaggagacttcaattaggtataaataccagcagccagaggaggtgcagcacattgttctgatcatctgaagatcagctattagaagagaaagatcagttaagtcctttgg

SEQ ID NO: 21 - DNA, 47 bp, synthetic construct
  source 1..47: mol_type = other DNA; note = minCMV promoter
cctatataagcagagctcgtttagtgaaccgtcagatcgcctggaga

SEQ ID NO: 22 - DNA, 427 bp, synthetic construct
  source 1..427: mol_type = other DNA; note = pGM-CSF-minCMV promoter
taagtgtctcccacgccccaccccagccattccaggccaggaagtccaaactgtgcccctcagagggagggggcagcctcaggcccattcagactgcccagggagggctggagagccctcaggaaggcgggtgggtgggctgtcggttcttggaaaggttcattaatgaaaacccccaagcctgaccacctagggaaaaggctcaccgttcccatgtgtggctgataagggccaggagattccacagttcaggtagttcccccgcctccctggcattttgtggtcaccattaatcatttcctctgtgtatttaagagctcttttgccagtgagcccagtacacagagagaaaggctaaagttctctggaggagcggccgccctatataagcagagctcgtttagtgaaccgtcagatcgcctggaga

SEQ ID NO: 23 - DNA, 390 bp, synthetic construct
  source 1..390: mol_type = other DNA; note = pGM-CSF-minCMV promoter
taagtgtctcccacgccccaccccagccattccaggccaggaagtccaaactgtgcccctcagagggagggggcagcctcaggcccattcagactgcccagggagggctggagagccctcaggaaggcgggtgggtgggctgtcggttcttggaaaggttcattaatgaaaacccccaagcctgaccacctagggaaaaggctcaccgttcccatgtgtggctgataagggccaggagattccacagttcaggtagttcccccgcctccctggcattttgtggtcaccattaatcatttcctctgtgtatttaagagctcttttgccagtgagccgcggccgccctatataagcagagctcgtttagtgaaccgtcagatcgcctggaga

SEQ ID NO: 24 - DNA, 357 bp, synthetic construct
  source 1..357: mol_type = other DNA; note = pGM-CSF-minCMV promoter
taagtgtctcccacgccccaccccagccattccaggccaggaagtccaaactgtgcccctcagagggagggggcagcctcaggcccattcagactgcccagggagggctggagagccctcaggaaggcgggtgggtgggctgtcggttcttggaaaggttcattaatgaaaacccccaagcctgaccacctagggaaaaggctcaccgttcccatgtgtggctgataagggccaggagattccacagttcaggtagttcccccgcctccctggcattttgtggtcaccattaatcatttcctgcggccgccctatataagcagagctcgtttagtgaaccgtcagatcgcctggaga

SEQ ID NO: 25 - DNA, 271 bp, synthetic construct
  source 1..271: mol_type = other DNA; note = pGM-CSF-minCMV promoter
caggaaggcgggtgggtgggctgtcggttcttggaaaggttcattaatgaaaacccccaagcctgaccacctagggaaaaggctcaccgttcccatgtgtggctgataagggccaggagattccacagttcaggtagttcccccgcctccctggcattttgtggtcaccattaatcatttcctctgtgtatttaagagctcttttgccagtgagccgcggccgccctatataagcagagctcgtttagtgaaccgtcagatcgcctggaga

SEQ ID NO: 26 - DNA, 238 bp, synthetic construct
  source 1..238: mol_type = other DNA; note = pGM-CSF-minCMV promoter
caggaaggcgggtgggtgggctgtcggttcttggaaaggttcattaatgaaaacccccaagcctgaccacctagggaaaaggctcaccgttcccatgtgtggctgataagggccaggagattccacagttcaggtagttcccccgcctccctggcattttgtggtcaccattaatcatttcctgcggccgccctatataagcagagctcgtttagtgaaccgtcagatcgcctggaga

SEQ ID NO: 27 - DNA, 200 bp, synthetic construct
  source 1..200: mol_type = other DNA; note = pGM-CSF-minCMV promoter
gttcattaatgaaaacccccaagcctgaccacctagggaaaaggctcaccgttcccatgtgtggctgataagggccaggagattccacagttcaggtagttcccccgcctccctggcattttgtggtcaccattaatcatttcctgcggccgccctatataagcagagctcgtttagtgaaccgtcagatcgcctggaga

SEQ ID NO: 28 - DNA, 127 bp, synthetic construct
  source 1..127: mol_type = other DNA; note = pGM-CSF-minCMV promoter
gccaggagattccacagttcaggtagttcccccgcctccctggcattttgtggtcaccattaatcatttcctgcggccgccctatataagcagagctcgtttagtgaaccgtcagatcgcctggaga

SEQ ID NO: 29 - DNA, 308 bp, synthetic construct
  source 1..308: mol_type = other DNA; note = pGM-CSF-minCMV promoter
caggaaggcgggtgggtgggctgtcggttcttggaaaggttcattaatgaaaacccccaagcctgaccacctagggaaaaggctcaccgttcccatgtgtggctgataagggccaggagattccacagttcaggtagttcccccgcctccctggcattttgtggtcaccattaatcatttcctctgtgtatttaagagctcttttgccagtgagcccagtacacagagagaaaggctaaagttctctggaggagcggccgccctatataagcagagctcgtttagtgaaccgtcagatcgcctggaga

SEQ ID NO: 30 - DNA, 353 bp, synthetic construct
  source 1..353: mol_type = other DNA; note = 6*NFAT-minIL2 promoter
ggaggaaaaactgtttcatacagaaggcgtcaattaggaggaaaaactgtttcatacagaaggcgtcaattaggaggaaaaactgtttcatacagaaggcgtcaattggtcccatcgaattaggaggaaaaactgtttcatacagaaggcgtcaattaggaggaaaaactgtttcatacagaaggcgtcaattaggaggaaaaactgtttcatacagaaggcgtcaattggtcccgggacattttgacacccccataatatttttccagaattaacagtataaattgcatctcttgttcaagagttccctatcactctctttaatcactactcacagtaacctcaactcctga

SEQ ID NO: 31 - DNA, 49 bp, synthetic construct
  source 1..49: mol_type = other DNA; note = bidirectional poly A
aataaaatatctttattttcattacatctgtgtgttggttttttgtgtg